European Patent Specification EP 3 371 309 B1, published July 5, 2023. Title: COMBINATORIAL SETS OF NUCLEIC ACID BARCODES FOR ANALYSIS OF NUCLEIC ACIDS ASSOCIATED WITH SINGLE CELLS. Applicant: Atreca, Inc. The sequence listing filed with the application follows.

SEQUENCE LISTING (6 sequences)

SEQ ID NO: 1 - DNA, 51 bp, artificial sequence
  synthetic construct
  misc_feature (27)..(34): n is a, c, g, or t
ggctcggagatgtgtataagagacagnnnnnnnnttttttttttttttttv

SEQ ID NO: 2 - DNA, 30 bp, artificial sequence
  synthetic construct
ggaagatagggataacagggtaatgacggg

SEQ ID NO: 3 - DNA, 65 bp, artificial sequence
  synthetic construct
aatgatacggcgaccaccgagatctacactcgtcggcagcggaagatagggataacagggtaatg

SEQ ID NO: 4 - DNA, 55 bp, artificial sequence
  synthetic construct
caagcagaagacggcatacgagatgtctcgtgggctcggagatgtgtataagaga

SEQ ID NO: 5 - DNA, 17 bp, artificial sequence
  synthetic construct
aatgatacggcgaccac

SEQ ID NO: 6 - DNA, 19 bp, artificial sequence
  synthetic construct
caagcagaagacggcatac